European Patent Application EP 4 174 493 A1, published May 3, 2023. Title: Method of predicting a patient's benefit from therapy with an immune checkpoint inhibitor. Applicant: Eberhard Karls Universität Tübingen, Medizinische Fakultät. The sequence listing filed with the application follows.

SEQUENCE LISTING (14 sequences)

SEQ ID NO: 1 - DNA, 20 bp, Artificial sequence
  PCR primer
accgtgggcaactctgtcaa

SEQ ID NO: 2 - DNA, 20 bp, Artificial sequence
  PCR primer
cccactcatctccaacggca

SEQ ID NO: 3 - DNA, 20 bp, Artificial sequence
  PCR primer
ggcacgggtcttctcctacc

SEQ ID NO: 4 - DNA, 21 bp, Artificial sequence
  PCR primer
tgtccgaggtttgtctccagg

SEQ ID NO: 5 - DNA, 20 bp, Artificial sequence
  PCR primer
cctgcaccgacatggaggat

SEQ ID NO: 6 - DNA, 20 bp, Artificial sequence
  PCR primer
cgtaagtgaagcccgaccga

SEQ ID NO: 7 - DNA, 21 bp, Artificial sequence
  PCR primer
tgaaacgactggaggtggaca

SEQ ID NO: 8 - DNA, 21 bp, Artificial sequence
  PCR primer
cacgagctaaagccctactgc

SEQ ID NO: 9 - DNA, 20 bp, Artificial sequence
  PCR primer
tcgacagtcagccgcatctt

SEQ ID NO: 10 - DNA, 21 bp, Artificial sequence
  PCR primer
gcccaatacgaccaaatccgt

SEQ ID NO: 11 - protein, 9 aa, Artificial sequence
  None
YVLDHLIVV

SEQ ID NO: 12 - protein, 9 aa, Artificial sequence
  None
NLVPMVATV

SEQ ID NO: 13 - protein, 9 aa, Artificial sequence
  None
KLFEKVKEV

SEQ ID NO: 14 - protein, 9 aa, Artificial sequence
  None
KPSEKIQVL